European Patent Specification EP 3 600 429 B1, published October 25, 2023. Title: IL-37 FUSION PROTEIN AND METHODS OF MAKING AND USING SAME. Applicant: BIO-TECHNE CORPORATION THE REGENTS OF THE UNIVERSITY OF COLORADO KALABOKIS, Vassilios DINARELLO, Charles A. The sequence listing filed with the application follows.

SEQUENCE LISTING (14 sequences)

SEQ ID NO: 1 - protein, 173 aa, Homo sapiens
VHTSPKVKNLNPKKFSIHDQDHKVLVLDSGNLIAVPDKNYIRPEIFFALASSLSSASAEKGSPILLGVSKGEFCLYCDKDKGQSHPSLQLKKEKLMKLAAQKESARRPFIFYRAQVGSWNMLESAAHPGWFICTSCNCNEPVGVTDKFENRKHIEFSFQPVCKAEMSPSEVSD

SEQ ID NO: 2 - protein, 161 aa, Homo sapiens
VHTSPKVKNLNPKKFSIHDQDHKVLVLDSGNLIAVPDKNYIRPEIFFALASSLSSASAEKGSPILLGVSKGEFCLYCDKDKGQSHPSLQLKKEKLMKLAAQKESARRPFIFYRAQVGSWNMLESAAHPGWFICTSCNCNEPVGVTDKFENRKHIEFSFQPV

SEQ ID NO: 3 - protein, 154 aa, Homo sapiens
KNLNPKKFSIHDQDHKVLVLDSGNLIAVPDKNYIRPEIFFALASSLSSASAEKGSPILLGVSKGEFCLYCDKDKGQSHPSLQLKKEKLMKLAAQKESARRPFIFYRAQVGSWNMLESAAHPGWFICTSCNCNEPVGVTDKFENRKHIEFSFQPV

SEQ ID NO: 4 - protein, 231 aa, Homo sapiens
PKSCDKTHTCPPCPAPEAEGAPSVFLFPPKPKDTLMISRTPEVTCVVVDVSHEDPEVKFNWYVDGVEVHNAKTKPREEQYNSTYRVVSVLTVLHQDWLNGKEYKCKVSNKALPAPIEKTISKAKGQPREPQVYTLPPSRDELTKNQVSLTCLVKGFYPSDIAVEWESNGQPENNYKATPPVLDSDGSFFLYSKLTVDKSRWQQGNVFSCSVMHEALHNHYTQKSLSLSPGK

SEQ ID NO: 5 - protein, 231 aa, artificial
  non-lytic hIgG1-Fc sequence
PKSCDKTHTCPPCPAPEAEGAPSVFLFPPKPKDTLMISRTPEVTCVVVDVSHEDPEVKFNWYVDGVEVHNAKTKPREEQYNSTYRVVSVLTVLHQDWLNGKAYACAVSNKALPAPIEKTISKAKGQPREPQVYTLPPSRDELTKNQVSLTCLVKGFYPSDIAVEWESNGQPENNYKATPPVLDSDGSFFLYSKLTVDKSRWQQGNVFSCSVMHEALHNHYTQKSLSLSPGK

SEQ ID NO: 6 - protein, 16 aa, artificial
  CD33 signal sequence
MPLLLLLPLLWAGALA

SEQ ID NO: 7 - protein, 396 aa, artificial
  human IL-37 Fc aa46-206
VHTSPKVKNLNPKKFSIHDQDHKVLVLDSGNLIAVPDKNYIRPEIFFALASSLSSASAEKGSPILLGVSKGEFCLYCDKDKGQSHPSLQLKKEKLMKLAAQKESARRPFIFYRAQVGSWNMLESAAHPGWFICTSCNCNEPVGVTDKFENRKHIEFSFQPVGGGSPKSCDKTHTCPPCPAPEAEGAPSVFLFPPKPKDTLMISRTPEVTCVVVDVSHEDPEVKFNWYVDGVEVHNAKTKPREEQYNSTYRVVSVLTVLHQDWLNGKEYKCKVSNKALPAPIEKTISKAKGQPREPQVYTLPPSRDELTKNQVSLTCLVKGFYPSDIAVEWESNGQPENNYKATPPVLDSDGSFFLYSKLTVDKSRWQQGNVFSCSVMHEALHNHYTQKSLSLSPGK

SEQ ID NO: 8 - protein, 389 aa, artificial
  human IL-37 Fc aa53-206
KNLNPKKFSIHDQDHKVLVLDSGNLIAVPDKNYIRPEIFFALASSLSSASAEKGSPILLGVSKGEFCLYCDKDKGQSHPSLQLKKEKLMKLAAQKESARRPFIFYRAQVGSWNMLESAAHPGWFICTSCNCNEPVGVTDKFENRKHIEFSFQPVGGGSPKSCDKTHTCPPCPAPEAEGAPSVFLFPPKPKDTLMISRTPEVTCVVVDVSHEDPEVKFNWYVDGVEVHNAKTKPREEQYNSTYRVVSVLTVLHQDWLNGKEYKCKVSNKALPAPIEKTISKAKGQPREPQVYTLPPSRDELTKNQVSLTCLVKGFYPSDIAVEWESNGQPENNYKATPPVLDSDGSFFLYSKLTVDKSRWQQGNVFSCSVMHEALHNHYTQKSLSLSPGK

SEQ ID NO: 9 - protein, 192 aa, Homo sapiens
MSGCDRRETETKGKNSFKKRLRGPKVKNLNPKKFSIHDQDHKVLVLDSGNLIAVPDKNYIRPEIFFALASSLSSASAEKGSPILLGVSKGEFCLYCDKDKGQSHPSLQLKKEKLMKLAAQKESARRPFIFYRAQVGSWNMLESAAHPGWFICTSCNCNEPVGVTDKFENRKHIEFSFQPVCKAEMSPSEVSD

SEQ ID NO: 10 - protein, 218 aa, Homo sapiens
MSFVGENSGVKMGSEDWEKDEPQCCLEDPAGSPLEPGPSLPTMNFVHTSPKVKNLNPKKFSIHDQDHKVLVLDSGNLIAVPDKNYIRPEIFFALASSLSSASAEKGSPILLGVSKGEFCLYCDKDKGQSHPSLQLKKEKLMKLAAQKESARRPFIFYRAQVGSWNMLESAAHPGWFICTSCNCNEPVGVTDKFENRKHIEFSFQPVCKAEMSPSEVSD

SEQ ID NO: 11 - protein, 178 aa, Homo sapiens
MSFVGENSGVKMGSEDWEKDEPQCCLEDPAGSPLEPGPSLPTMNFVHTEIFFALASSLSSASAEKGSPILLGVSKGEFCLYCDKDKGQSHPSLQLKKEKLMKLAAQKESARRPFIFYRAQVGSWNMLESAAHPGWFICTSCNCNEPVGVTDKFENRKHIEFSFQPVCKAEMSPSEVSD

SEQ ID NO: 12 - protein, 197 aa, Homo sapiens
MSFVGENSGVKMGSEDWEKDEPQCCLEGPKVKNLNPKKFSIHDQDHKVLVLDSGNLIAVPDKNYIRPEIFFALASSLSSASAEKGSPILLGVSKGEFCLYCDKDKGQSHPSLQLKKEKLMKLAAQKESARRPFIFYRAQVGSWNMLESAAHPGWFICTSCNCNEPVGVTDKFENRKHIEFSFQPVCKAEMSPSEVSD

SEQ ID NO: 13 - protein, 157 aa, Homo sapiens
MSFVGENSGVKMGSEDWEKDEPQCCLEEIFFALASSLSSASAEKGSPILLGVSKGEFCLYCDKDKGQSHPSLQLKKEKLMKLAAQKESARRPFIFYRAQVGSWNMLESAAHPGWFICTSCNCNEPVGVTDKFENRKHIEFSFQPVCKAEMSPSEVSD

SEQ ID NO: 14 - protein, 412 aa, artificial
  CD33 signal sequence and human IL-37 Fc aa46-206
MPLLLLLPLLWAGALAVHTSPKVKNLNPKKFSIHDQDHKVLVLDSGNLIAVPDKNYIRPEIFFALASSLSSASAEKGSPILLGVSKGEFCLYCDKDKGQSHPSLQLKKEKLMKLAAQKESARRPFIFYRAQVGSWNMLESAAHPGWFICTSCNCNEPVGVTDKFENRKHIEFSFQPVGGGSPKSCDKTHTCPPCPAPEAEGAPSVFLFPPKPKDTLMISRTPEVTCVVVDVSHEDPEVKFNWYVDGVEVHNAKTKPREEQYNSTYRVVSVLTVLHQDWLNGKEYKCKVSNKALPAPIEKTISKAKGQPREPQVYTLPPSRDELTKNQVSLTCLVKGFYPSDIAVEWESNGQPENNYKATPPVLDSDGSFFLYSKLTVDKSRWQQGNVFSCSVMHEALHNHYTQKSLSLSPGK